European Patent Application EP 4 785 935 A1, published August 5, 2026. Title: 一种来源于细胞内的靶向纳米囊泡的制备方法和应用. Applicant: 天津医科大学眼科医院. The sequence listing filed with the application follows.

SEQUENCE LISTING (4 sequences)

SEQ ID NO: 1 - DNA, 1248 bp, synthetic construct
  source 1..1248: mol_type = other DNA
atggtgtgcttccgcctcttcccggttccgggctcagggctcgttctggtctgcctagtcctgggagctgtgcggtcttatgcagagagcgaggaggaggacttggaacttaatttgacagattcagaaaatgccacttgcctttatgcaaaatggcagatgaatttcacagtacgctatgaaactacaaataaaacttataaaactgtaaccatttcagaccatggcactgtgacatataatggaagcatttgtggggatgatcagaatggtcccaaaatagcagtgcagttcggacctggcttttcctggattgcgaattttaccaaggcagcatctacttattcaattgacagcgtctcattttcctacaacactggtgataacacaacatttcctgatgctgaagataaaggaattcttactgttgatgaacttttggccatcagaattccattgaatgacctttttagatgcaatagtttatcaactttggaaaagaatgatgttgtccaacactactgggatgttcttgtacaagcttttgtccaaaatggcacagtgagcacaaatgagttcctgtgtgataaagacaaaacttcaacagtggcacccaccatacacaccactgtgccatctcctactacaacacctactccaaaggaaaaaccagaagctggaacctattcagttaataatggcaatgatacttgtctgctggctaccatggggctgcagctgaacatcactcaggataaggttgcttcagttattaacatcaaccccaatacaactcactccacaggcagctgccgttctcacactgctctacttagactcaatagcagcaccattaagtatctagactttgtctttgctgtgaaaaatgaaaaccgattttatctgaaggaagtgaacatcagcatgtatttggttaatggctccgttttcagcattgcaaataacaatctcagctactgggatgcccccctgggaagttcttatatgtgcaacaaagagcagactgtttcagtgtctggagcatttcagataaatacctttgatctaagggttcagcctttcaatgtgacacaaggaaagtattctacagcccaagagtgttcgctggatgatgacaccattctaatcccaattatagttggtgctggtctttcaggcttgattatcgttatagtgattgcttacgtaattggcagaagaaaaagttatgctggatatcagactctg

SEQ ID NO: 2 - DNA, 20 bp, synthetic construct
  source 1..20: mol_type = other DNA
tggctccgttttcagcattg

SEQ ID NO: 3 - DNA, 20 bp, synthetic construct
  source 1..20: mol_type = other DNA
tggtgtcatcatccagcgaa

SEQ ID NO: 4 - protein, 8 aa, synthetic construct
DYKDDDDK